European Patent Specification EP 3 390 451 B1, published January 22, 2025. Title: Caninized Human Antibodies to Human IL- 4R alpha. Applicant: Intervet Inc. Intervet International BV. Morsey, Mohamad A Zhang, Yuanzheng. The sequence listing filed with the application follows.

SEQUENCE LISTING (94 sequences)

SEQ ID NO: 1 - DNA, 2469 bp, Canis familiaris
atgggcagactgtgcagcggcctgaccttccccgtgagctgcctggtgctggtgtgggtggccagcagcggcagcgtgaaggtgctgcacgagcccagctgcttcagcgactacatcagcaccagcgtgtgccagtggaagatggaccaccccaccaactgcagcgccgagctgagactgagctaccagctggacttcatgggcagcgagaaccacacctgcgtgcccgagaacagagaggacagcgtgtgcgtgtgcagcatgcccatcgacgacgccgtggaggccgacgtgtaccagctggacctgtgggccggccagcagctgctgtggagcggcagcttccagcccagcaagcacgtgaagcccagaacccccggcaacctgaccgtgcaccccaacatcagccacacctggctgctgatgtggaccaacccctaccccaccgagaaccacctgcacagcgagctgacctacatggtgaacgtgagcaacgacaacgaccccgaggacttcaaggtgtacaacgtgacctacatgggccccaccctgagactggccgccagcaccctgaagagcggcgccagctacagcgccagagtgagagcctgggcccagacctacaacagcacctggagcgactggagccccagcaccacctggctgaactactacgagccctgggagcagcacctgcccctgggcgtgagcatcagctgcctggtgatcctggccatctgcctgagctgctacttcagcatcatcaagatcaagaagggctggtgggaccagatccccaaccccgcccacagccccctggtggccatcgtgatccaggacagccaggtgagcctgtggggcaagagaagcagaggccaggagcccgccaagtgcccccactggaagacctgcctgaccaagctgctgccctgcctgctggagcacggcctgggcagagaggaggagagccccaagaccgccaagaacggccccctgcagggccccggcaagcccgcctggtgccccgtggaggtgagcaagaccatcctgtggcccgagagcatcagcgtggtgcagtgcgtggagctgagcgaggcccccgtggacaacgaggaggaggaggaggtggaggaggacaagagaagcctgtgccccagcctggagggcagcggcggcagcttccaggagggcagagagggcatcgtggccagactgaccgagagcctgttcctggacctgctgggcggcgagaacggcggcttctgcccccagggcctggaggagagctgcctgcccccccccagcggcagcgtgggcgcccagatgccctgggcccagttccccagagccggccccagagccgcccccgagggccccgagcagcccagaagacccgagagcgccctgcaggccagccccacccagagcgccggcagcagcgccttccccgagcccccccccgtggtgaccgacaaccccgcctacagaagcttcggcagcttcctgggccagagcagcgaccccggcgacggcgacagcgaccccgagctggccgacagacccggcgaggccgaccccggcatccccagcgccccccagccccccgagccccccgccgccctgcagcccgagcccgagagctgggagcagatcctgagacagagcgtgctgcagcacagagccgcccccgcccccggccccggccccggcagcggctacagagagttcacctgcgccgtgaagcagggcagcgcccccgacgccggcggccccggcttcggccccagcggcgaggccggctacaaggccttctgcagcctgctgcccggcggcgccacctgccccggcaccagcggcggcgaggccggcagcggcgagggcggctacaagcccttccagagcctgacccccggctgccccggcgcccccacccccgtgcccgtgcccctgttcaccttcggcctggacaccgagccccccggcagcccccaggacagcctgggcgccggcagcagccccgagcacctgggcgtggagcccgccggcaaggaggaggacagcagaaagaccctgctggcccccgagcaggccaccgaccccctgagagacgacctggccagcagcatcgtgtacagcgccctgacctgccacctgtgcggccacctgaagcagtggcacgaccaggaggagagaggcaaggcccacatcgtgcccagcccctgctgcggctgctgctgcggcgacagaagcagcctgctgctgagccccctgagagcccccaacgtgctgcccggcggcgtgctgctggaggccagcctgagccccgccagcctggtgcccagcggcgtgagcaaggagggcaagagcagccccttcagccagcccgccagcagcagcgcccagagcagcagccagacccccaagaagctggccgtgctgagcaccgagcccacctgcatgagcgccagc

SEQ ID NO: 2 - protein, 823 aa, Canis familiaris
MGRLCSGLTFPVSCLVLVWVASSGSVKVLHEPSCFSDYISTSVCQWKMDHPTNCSAELRLSYQLDFMGSENHTCVPENREDSVCVCSMPIDDAVEADVYQLDLWAGQQLLWSGSFQPSKHVKPRTPGNLTVHPNISHTWLLMWTNPYPTENHLHSELTYMVNVSNDNDPEDFKVYNVTYMGPTLRLAASTLKSGASYSARVRAWAQTYNSTWSDWSPSTTWLNYYEPWEQHLPLGVSISCLVILAICLSCYFSIIKIKKGWWDQIPNPAHSPLVAIVIQDSQVSLWGKRSRGQEPAKCPHWKTCLTKLLPCLLEHGLGREEESPKTAKNGPLQGPGKPAWCPVEVSKTILWPESISVVQCVELSEAPVDNEEEEEVEEDKRSLCPSLEGSGGSFQEGREGIVARLTESLFLDLLGGENGGFCPQGLEESCLPPPSGSVGAQMPWAQFPRAGPRAAPEGPEQPRRPESALQASPTQSAGSSAFPEPPPVVTDNPAYRSFGSFLGQSSDPGDGDSDPELADRPGEADPGIPSAPQPPEPPAALQPEPESWEQILRQSVLQHRAAPAPGPGPGSGYREFTCAVKQGSAPDAGGPGFGPSGEAGYKAFCSLLPGGATCPGTSGGEAGSGEGGYKPFQSLTPGCPGAPTPVPVPLFTFGLDTEPPGSPQDSLGAGSSPEHLGVEPAGKEEDSRKTLLAPEQATDPLRDDLASSIVYSALTCHLCGHLKQWHDQEERGKAHIVPSPCCGCCCGDRSSLLLSPLRAPNVLPGGVLLEASLSPASLVPSGVSKEGKSSPFSQPASSSAQSSSQTPKKLAVLSTEPTCMSAS

SEQ ID NO: 3 - DNA, 2394 bp, Canis familiaris
gtgaaggtgctgcacgagcccagctgcttcagcgactacatcagcaccagcgtgtgccagtggaagatggaccaccccaccaactgcagcgccgagctgagactgagctaccagctggacttcatgggcagcgagaaccacacctgcgtgcccgagaacagagaggacagcgtgtgcgtgtgcagcatgcccatcgacgacgccgtggaggccgacgtgtaccagctggacctgtgggccggccagcagctgctgtggagcggcagcttccagcccagcaagcacgtgaagcccagaacccccggcaacctgaccgtgcaccccaacatcagccacacctggctgctgatgtggaccaacccctaccccaccgagaaccacctgcacagcgagctgacctacatggtgaacgtgagcaacgacaacgaccccgaggacttcaaggtgtacaacgtgacctacatgggccccaccctgagactggccgccagcaccctgaagagcggcgccagctacagcgccagagtgagagcctgggcccagacctacaacagcacctggagcgactggagccccagcaccacctggctgaactactacgagccctgggagcagcacctgcccctgggcgtgagcatcagctgcctggtgatcctggccatctgcctgagctgctacttcagcatcatcaagatcaagaagggctggtgggaccagatccccaaccccgcccacagccccctggtggccatcgtgatccaggacagccaggtgagcctgtggggcaagagaagcagaggccaggagcccgccaagtgcccccactggaagacctgcctgaccaagctgctgccctgcctgctggagcacggcctgggcagagaggaggagagccccaagaccgccaagaacggccccctgcagggccccggcaagcccgcctggtgccccgtggaggtgagcaagaccatcctgtggcccgagagcatcagcgtggtgcagtgcgtggagctgagcgaggcccccgtggacaacgaggaggaggaggaggtggaggaggacaagagaagcctgtgccccagcctggagggcagcggcggcagcttccaggagggcagagagggcatcgtggccagactgaccgagagcctgttcctggacctgctgggcggcgagaacggcggcttctgcccccagggcctggaggagagctgcctgcccccccccagcggcagcgtgggcgcccagatgccctgggcccagttccccagagccggccccagagccgcccccgagggccccgagcagcccagaagacccgagagcgccctgcaggccagccccacccagagcgccggcagcagcgccttccccgagcccccccccgtggtgaccgacaaccccgcctacagaagcttcggcagcttcctgggccagagcagcgaccccggcgacggcgacagcgaccccgagctggccgacagacccggcgaggccgaccccggcatccccagcgccccccagccccccgagccccccgccgccctgcagcccgagcccgagagctgggagcagatcctgagacagagcgtgctgcagcacagagccgcccccgcccccggccccggccccggcagcggctacagagagttcacctgcgccgtgaagcagggcagcgcccccgacgccggcggccccggcttcggccccagcggcgaggccggctacaaggccttctgcagcctgctgcccggcggcgccacctgccccggcaccagcggcggcgaggccggcagcggcgagggcggctacaagcccttccagagcctgacccccggctgccccggcgcccccacccccgtgcccgtgcccctgttcaccttcggcctggacaccgagccccccggcagcccccaggacagcctgggcgccggcagcagccccgagcacctgggcgtggagcccgccggcaaggaggaggacagcagaaagaccctgctggcccccgagcaggccaccgaccccctgagagacgacctggccagcagcatcgtgtacagcgccctgacctgccacctgtgcggccacctgaagcagtggcacgaccaggaggagagaggcaaggcccacatcgtgcccagcccctgctgcggctgctgctgcggcgacagaagcagcctgctgctgagccccctgagagcccccaacgtgctgcccggcggcgtgctgctggaggccagcctgagccccgccagcctggtgcccagcggcgtgagcaaggagggcaagagcagccccttcagccagcccgccagcagcagcgcccagagcagcagccagacccccaagaagctggccgtgctgagcaccgagcccacctgcatgagcgccagc

SEQ ID NO: 4 - protein, 798 aa, Canis familiaris
VKVLHEPSCFSDYISTSVCQWKMDHPTNCSAELRLSYQLDFMGSENHTCVPENREDSVCVCSMPIDDAVEADVYQLDLWAGQQLLWSGSFQPSKHVKPRTPGNLTVHPNISHTWLLMWTNPYPTENHLHSELTYMVNVSNDNDPEDFKVYNVTYMGPTLRLAASTLKSGASYSARVRAWAQTYNSTWSDWSPSTTWLNYYEPWEQHLPLGVSISCLVILAICLSCYFSIIKIKKGWWDQIPNPAHSPLVAIVIQDSQVSLWGKRSRGQEPAKCPHWKTCLTKLLPCLLEHGLGREEESPKTAKNGPLQGPGKPAWCPVEVSKTILWPESISVVQCVELSEAPVDNEEEEEVEEDKRSLCPSLEGSGGSFQEGREGIVARLTESLFLDLLGGENGGFCPQGLEESCLPPPSGSVGAQMPWAQFPRAGPRAAPEGPEQPRRPESALQASPTQSAGSSAFPEPPPVVTDNPAYRSFGSFLGQSSDPGDGDSDPELADRPGEADPGIPSAPQPPEPPAALQPEPESWEQILRQSVLQHRAAPAPGPGPGSGYREFTCAVKQGSAPDAGGPGFGPSGEAGYKAFCSLLPGGATCPGTSGGEAGSGEGGYKPFQSLTPGCPGAPTPVPVPLFTFGLDTEPPGSPQDSLGAGSSPEHLGVEPAGKEEDSRKTLLAPEQATDPLRDDLASSIVYSALTCHLCGHLKQWHDQEERGKAHIVPSPCCGCCCGDRSSLLLSPLRAPNVLPGGVLLEASLSPASLVPSGVSKEGKSSPFSQPASSSAQSSSQTPKKLAVLSTEPTCMSAS

SEQ ID NO: 5 - DNA, 624 bp, Canis familiaris
gtgaaggtgctgcacgagcccagctgcttcagcgactacatcagcaccagcgtgtgccagtggaagatggaccaccccaccaactgcagcgccgagctgagactgagctaccagctggacttcatgggcagcgagaaccacacctgcgtgcccgagaacagagaggacagcgtgtgcgtgtgcagcatgcccatcgacgacgccgtggaggccgacgtgtaccagctggacctgtgggccggccagcagctgctgtggagcggcagcttccagcccagcaagcacgtgaagcccagaacccccggcaacctgaccgtgcaccccaacatcagccacacctggctgctgatgtggaccaacccctaccccaccgagaaccacctgcacagcgagctgacctacatggtgaacgtgagcaacgacaacgaccccgaggacttcaaggtgtacaacgtgacctacatgggccccaccctgagactggccgccagcaccctgaagagcggcgccagctacagcgccagagtgagagcctgggcccagacctacaacagcacctggagcgactggagccccagcaccacctggctgaactactacgagccctgggagcagcacctgccc

SEQ ID NO: 6 - protein, 208 aa, Canis familiaris
VKVLHEPSCFSDYISTSVCQWKMDHPTNCSAELRLSYQLDFMGSENHTCVPENREDSVCVCSMPIDDAVEADVYQLDLWAGQQLLWSGSFQPSKHVKPRTPGNLTVHPNISHTWLLMWTNPYPTENHLHSELTYMVNVSNDNDPEDFKVYNVTYMGPTLRLAASTLKSGASYSARVRAWAQTYNSTWSDWSPSTTWLNYYEPWEQHLP

SEQ ID NO: 7 - DNA, 648 bp, Artificial Sequence
  Canis familiaris plus His Tag
gtgaaggtgctgcacgagcccagctgcttcagcgactacatcagcaccagcgtgtgccagtggaagatggaccaccccaccaactgcagcgccgagctgagactgagctaccagctggacttcatgggcagcgagaaccacacctgcgtgcccgagaacagagaggacagcgtgtgcgtgtgcagcatgcccatcgacgacgccgtggaggccgacgtgtaccagctggacctgtgggccggccagcagctgctgtggagcggcagcttccagcccagcaagcacgtgaagcccagaacccccggcaacctgaccgtgcaccccaacatcagccacacctggctgctgatgtggaccaacccctaccccaccgagaaccacctgcacagcgagctgacctacatggtgaacgtgagcaacgacaacgaccccgaggacttcaaggtgtacaacgtgacctacatgggccccaccctgagactggccgccagcaccctgaagagcggcgccagctacagcgccagagtgagagcctgggcccagacctacaacagcacctggagcgactggagccccagcaccacctggctgaactactacgagccctgggagcagcacctgccccaccaccaccaccaccaccaccac

SEQ ID NO: 8 - protein, 216 aa, Artificial Sequence
  Canis familiaris plus His Tag
VKVLHEPSCFSDYISTSVCQWKMDHPTNCSAELRLSYQLDFMGSENHTCVPENREDSVCVCSMPIDDAVEADVYQLDLWAGQQLLWSGSFQPSKHVKPRTPGNLTVHPNISHTWLLMWTNPYPTENHLHSELTYMVNVSNDNDPEDFKVYNVTYMGPTLRLAASTLKSGASYSARVRAWAQTYNSTWSDWSPSTTWLNYYEPWEQHLPHHHHHHHH

SEQ ID NO: 9 - DNA, 1317 bp, Artificial Sequence
  Canis familiaris plus human
gtgaaggtgctgcacgagcccagctgcttcagcgactacatcagcaccagcgtgtgccagtggaagatggaccaccccaccaactgcagcgccgagctgagactgagctaccagctggacttcatgggcagcgagaaccacacctgcgtgcccgagaacagagaggacagcgtgtgcgtgtgcagcatgcccatcgacgacgccgtggaggccgacgtgtaccagctggacctgtgggccggccagcagctgctgtggagcggcagcttccagcccagcaagcacgtgaagcccagaacccccggcaacctgaccgtgcaccccaacatcagccacacctggctgctgatgtggaccaacccctaccccaccgagaaccacctgcacagcgagctgacctacatggtgaacgtgagcaacgacaacgaccccgaggacttcaaggtgtacaacgtgacctacatgggccccaccctgagactggccgccagcaccctgaagagcggcgccagctacagcgccagagtgagagcctgggcccagacctacaacagcacctggagcgactggagccccagcaccacctggctgaactactacgagccctgggagcagcacctggagcccaagagctgcgacaagacccacacctgccccccctgccccgcccccgagctgctgggcggccccagcgtgttcctgttcccccccaagcccaaggacaccctgatgatcagcagaacccccgaggtgacctgcgtggtggtggacgtgagccacgaggaccccgaggtgaagttcaactggtacgtggacggcgtggaggtgcacaacgccaagaccaagcccagagaggagcagtacaacagcacctacagagtggtgagcgtgctgaccgtgctgcaccaggactggctgaacggcaaggagtacaagtgcaaggtgagcaacaaggccctgcccgcccccatcgagaagaccatcagcaaggccaagggccagcccagagagccccaggtgtacaccctgccccccagcagagacgagctgaccaagaaccaggtgagcctgacctgcctggtgaagggcttctaccccagcgacatcgccgtggagtgggagagcaacggccagcccgagaacaactacaagaccaccccccccgtgctggacagcgacggcagcttcttcctgtacagcaagctgaccgtggacaagagcagatggcagcagggcaacgtgttcagctgcagcgtgatgcacgaggccctgcacaaccactacacccagaagagcctgagcctgagccccggcaag

SEQ ID NO: 10 - protein, 439 aa, Artificial Sequence
  Canis familiaris plus human
VKVLHEPSCFSDYISTSVCQWKMDHPTNCSAELRLSYQLDFMGSENHTCVPENREDSVCVCSMPIDDAVEADVYQLDLWAGQQLLWSGSFQPSKHVKPRTPGNLTVHPNISHTWLLMWTNPYPTENHLHSELTYMVNVSNDNDPEDFKVYNVTYMGPTLRLAASTLKSGASYSARVRAWAQTYNSTWSDWSPSTTWLNYYEPWEQHLEPKSCDKTHTCPPCPAPELLGGPSVFLFPPKPKDTLMISRTPEVTCVVVDVSHEDPEVKFNWYVDGVEVHNAKTKPREEQYNSTYRVVSVLTVLHQDWLNGKEYKCKVSNKALPAPIEKTISKAKGQPREPQVYTLPPSRDELTKNQVSLTCLVKGFYPSDIAVEWESNGQPENNYKTTPPVLDSDGSFFLYSKLTVDKSRWQQGNVFSCSVMHEALHNHYTQKSLSLSPGK

SEQ ID NO: 11 - protein, 336 aa, Canis familiaris
SASTTAPSVFPLAPSCGSTSGSTVALACLVSGYFPEPVTVSWNSGSLTSGVHTFPSVLQSSGLYSLSSMVTVPSSRWPSETFTCNVAHPASKTKVDKPVPKRENGRVPRPPDCPKCPAPEMLGGPSVFIFPPKPKDTLLIARTPEVTCVVVDLDPEDPEVQISWFVDGKQMQTAKTQPREEQFNGTYRVVSVLPIGHQDWLKGKQFTCKVNNKALPSPIERTISKARGQAHQPSVYVLPPSREELSKNTVSLTCLIKDFFPPDIDVEWQSNGQQEPESKYRTTPPQLDEDGSYFLYSKLSVDKSRWQRGDTFICAVMHEALHNHYTQESLSHSPGK

SEQ ID NO: 12 - protein, 331 aa, Artificial Sequence
  modified Canis familiaris
SASTTAPSVFPLAPSCGSTSGSTVALACLVSGYFPEPVTVSWNSGSLTSGVHTFPSVLQSSGLYSLSSMVTVPSSRWPSETFTCNVAHPASKTKVDKPVFNECRCTDTPPCPAPEMLGGPSVFIFPPKPKATLLIARTPEVTCVVVDLDPEDPEVQISWFVDGKQMQTAKTQPREEQFAGTYRVVSVLPIGHQDWLKGKQFTCKVNNKALPSPIERTISKARGQAHQPSVYVLPPSREELSKNTVSLTCLIKDFFPPDIDVEWQSNGQQEPESKYRTTPPQLDEDGSYFLYSKLSVDKSRWQRGDTFICAVMHEALHNHYTQESLSHSPGK

SEQ ID NO: 13 - protein, 331 aa, Artificial Sequence
  modified Canis familiaris
SASTTAPSVFPLAPSCGSTSGSTVALACLVSGYFPEPVTVSWNSGSLTSGVHTFPSVLQSSGLYSLSSMVTVPSSRWPSETFTCNVAHPASKTKVDKPVPKESTCKCISPCPAPEMLGGPSVFIFPPKPKATLLIARTPEVTCVVVDLDPEDPEVQISWFVDGKQMQTAKTQPREEQFAGTYRVVSVLPIGHQDWLKGKQFTCKVNNKALPSPIERTISKARGQAHQPSVYVLPPSREELSKNTVSLTCLIKDFFPPDIDVEWQSNGQQEPESKYRTTPPQLDEDGSYFLYSKLSVDKSRWQRGDTFICAVMHEALHNHYTQESLSHSPGK

SEQ ID NO: 14 - protein, 336 aa, Artificial Sequence
  modified Canis familiaris
SASTTAPSVFPLAPSCGSTSGSTVALACLVSGYFPEPVTVSWNSGSLTSGVHTFPSVLQSSGLYSLSSMVTVPSSRWPSETFTCNVAHPASKTKVDKPVPKRENGRVPRPPDCPKCPAPEMLGGPSVFIFPPKPKATLLIARTPEVTCVVVDLDPEDPEVQISWFVDGKQMQTAKTQPREEQFAGTYRVVSVLPIGHQDWLKGKQFTCKVNNKALPSPIERTISKARGQAHQPSVYVLPPSREELSKNTVSLTCLIKDFFPPDIDVEWQSNGQQEPESKYRTTPPQLDEDGSYFLYSKLSVDKSRWQRGDTFICAVMHEALHNHYTQESLSHSPGK

SEQ ID NO: 15 - DNA, 1380 bp, Artificial Sequence
  Canis familiaris plus human
gaggtgcagctggtggagtccggaggaggactggagcagcccggaggaagcctgagactgagctgcgctggcagcggcttcaccttcagggactacgccatgacctgggtgagacaggcccctggcaagggactggagtgggtgagcagcatcagcggctccggcggcaacacctactacgccgacagcgtgaagggcaggttcaccatcagcagggacaacagcaagaacaccctgtacctgcagatgaacagcctgagggccgaggacaccgccgtgtactactgcgccaaggaccgtttatctatcaccatcaggcccaggtactacggactggacgtgtggggccagggcaccacagtgaccgtgagcagcgcttccacaaccgcgccatcagtctttccgttggccccatcatgcgggtcgacgagcggatcgactgtggccctggcgtgcttggtgtcgggatactttcccgaacccgtcacggtcagctggaactccggatcgcttacgagcggtgtgcatacgttcccctcggtcttgcaatcatcagggctctactcgctgtcgagcatggtaacggtgccctcatcgaggtggccctccgaaacgttcacatgtaacgtagcacatccagcctccaaaaccaaggtggataaacccgtgccgaaaagagagaatgggcgggtgcctcgaccccctgattgccccaagtgtccggctccggaaatgctcggtggaccctcagtgtttatcttccctccgaagcccaaggacactctgctgatcgcgcgcactccagaagtaacatgtgtagtggtggcacttgatcccgaggaccccgaagtccagatctcctggtttgtagatgggaaacagatgcagaccgcaaaaactcaacccagagaggagcagttcgcaggaacataccgagtggtatccgtccttccgattggccaccaggactggttgaaagggaagcagtttacgtgtaaagtcaacaataaggcgttgcctagccctattgagcggacgatttcgaaagctaggggacaggcccaccagccatcggtctatgtccttccgccttcccgcgaggagctctcgaagaatacagtgagccttacatgcctcattaaggatttcttcccgcctgatatcgacgtagagtggcaatcaaacggtcaacaggagccggaatccaagtatagaaccactccgccccagcttgacgaggacggatcatactttttgtattcaaaactgtcggtggataagagccggtggcagagaggtgacaccttcatctgtgcggtgatgcacgaagcactccataatcactacacccaagagagcctctcgcattcccccggaaag

SEQ ID NO: 16 - protein, 460 aa, Artificial Sequence
  Canis familiaris plus human
EVQLVESGGGLEQPGGSLRLSCAGSGFTFRDYAMTWVRQAPGKGLEWVSSISGSGGNTYYADSVKGRFTISRDNSKNTLYLQMNSLRAEDTAVYYCAKDRLSITIRPRYYGLDVWGQGTTVTVSSASTTAPSVFPLAPSCGSTSGSTVALACLVSGYFPEPVTVSWNSGSLTSGVHTFPSVLQSSGLYSLSSMVTVPSSRWPSETFTCNVAHPASKTKVDKPVPKRENGRVPRPPDCPKCPAPEMLGGPSVFIFPPKPKDTLLIARTPEVTCVVVALDPEDPEVQISWFVDGKQMQTAKTQPREEQFAGTYRVVSVLPIGHQDWLKGKQFTCKVNNKALPSPIERTISKARGQAHQPSVYVLPPSREELSKNTVSLTCLIKDFFPPDIDVEWQSNGQQEPESKYRTTPPQLDEDGSYFLYSKLSVDKSRWQRGDTFICAVMHEALHNHYTQESLSHSPGK

SEQ ID NO: 17 - DNA, 669 bp, Artificial Sequence
  Canis familiaris plus human
gacatcgtgatgacccagagccccctgagcctgcctgtgacacctggcgagcctgccagcatcagctgcaggtccagccagagcctgctgtacagcatcggctacaactacctggactggtacctgcagaagagcggccagagcccccagctgctgatctacctgggcagcaatagagccagcggcgtgcccgatagatttagcggcagcggcagcggcacagacttcaccctgaagatcagcagggtggaggccgaggacgtgggcttctactactgcatgcaggccctgcagaccccctacaccttcggccagggcaccaagctggaaatcaagaggaacgacgctcagccagccgtgtacctcttccagccttcgccggaccagcttcatacggggtcagcgtcggtggtgtgcctgttgaactcgttttaccccaaggacattaacgtgaagtggaaggtagacggggtaattcaagacactggcattcaagagtccgtcacggaacaagactcaaaagactcaacgtattcactgtcgtcaaccttgacgatgtcaagcaccgagtatcttagccatgagctgtattcgtgcgagatcacccacaagtccctcccctccactcttatcaaatcctttcagcggtcggaatgtcagcgggtcgat

SEQ ID NO: 18 - protein, 223 aa, Artificial Sequence
  Canis familiaris plus human
DIVMTQSPLSLPVTPGEPASISCRSSQSLLYSIGYNYLDWYLQKSGQSPQLLIYLGSNRASGVPDRFSGSGSGTDFTLKISRVEAEDVGFYYCMQALQTPYTFGQGTKLEIKRNDAQPAVYLFQPSPDQLHTGSASVVCLLNSFYPKDINVKWKVDGVIQDTGIQESVTEQDSKDSTYSLSSTLTMSSTEYLSHELYSCEITHKSLPSTLIKSFQRSECQRVD

SEQ ID NO: 19 - DNA, 1353 bp, Artificial Sequence
  Canis familiaris plus human
caggtgcagctggtgcagagcggcgccgaagtgaagaagcctggcgccagcgtgaaggtgagctgcaaggccagcggctacgccttcaccagctactacatgcactgggccagacaggcccctggacagggactggagtggatgggcatcatcaaccctaggggcggcagcaccagctacgcccagaagttccagggcagggtggccatgaccagggacaccagcaccagcaccgtgtacatggaactgagcagcctgagacccgaggacaccgccgtgtactactgcgccaggggcaagtactggatgtacgactggggcaagggcaccctcgtgaccgtgagcagcgcttccacaaccgcgccatcagtctttccgttggccccatcatgcgggtcgacgagcggatcgactgtggccctggcgtgcttggtgtcgggatactttcccgaacccgtcacggtcagctggaactccggatcgcttacgagcggtgtgcatacgttcccctcggtcttgcaatcatcagggctctactcgctgtcgagcatggtaacggtgccctcatcgaggtggccctccgaaacgttcacatgtaacgtagcacatccagcctccaaaaccaaggtggataaacccgtgccgaaaagagagaatgggcgggtgcctcgaccccctgattgccccaagtgtccggctccggaaatgctcggtggaccctcagtgtttatcttccctccgaagcccaaggacactctgctgatcgcgcgcactccagaagtaacatgtgtagtggtggcacttgatcccgaggaccccgaagtccagatctcctggtttgtagatgggaaacagatgcagaccgcaaaaactcaacccagagaggagcagttcgcaggaacataccgagtggtatccgtccttccgattggccaccaggactggttgaaagggaagcagtttacgtgtaaagtcaacaataaggcgttgcctagccctattgagcggacgatttcgaaagctaggggacaggcccaccagccatcggtctatgtccttccgccttcccgcgaggagctctcgaagaatacagtgagccttacatgcctcattaaggatttcttcccgcctgatatcgacgtagagtggcaatcaaacggtcaacaggagccggaatccaagtatagaaccactccgccccagcttgacgaggacggatcatactttttgtattcaaaactgtcggtggataagagccggtggcagagaggtgacaccttcatctgtgcggtgatgcacgaagcactccataatcactacacccaagagagcctctcgcattcccccggaaag

SEQ ID NO: 20 - protein, 451 aa, Artificial Sequence
  Canis familiaris plus human
QVQLVQSGAEVKKPGASVKVSCKASGYAFTSYYMHWARQAPGQGLEWMGIINPRGGSTSYAQKFQGRVAMTRDTSTSTVYMELSSLRPEDTAVYYCARGKYWMYDWGKGTLVTVSSASTTAPSVFPLAPSCGSTSGSTVALACLVSGYFPEPVTVSWNSGSLTSGVHTFPSVLQSSGLYSLSSMVTVPSSRWPSETFTCNVAHPASKTKVDKPVPKRENGRVPRPPDCPKCPAPEMLGGPSVFIFPPKPKDTLLIARTPEVTCVVVALDPEDPEVQISWFVDGKQMQTAKTQPREEQFAGTYRVVSVLPIGHQDWLKGKQFTCKVNNKALPSPIERTISKARGQAHQPSVYVLPPSREELSKNTVSLTCLIKDFFPPDIDVEWQSNGQQEPESKYRTTPPQLDEDGSYFLYSKLSVDKSRWQRGDTFICAVMHEALHNHYTQESLSHSPGK

SEQ ID NO: 21 - DNA, 666 bp, Artificial Sequence
  Canis familiaris plus human
cagagcgtgctgacccagcctcctagcgtgagcgccgctcccggccagaaagtgaccatcagctgcagcggcggcggaagcagcatcggcaacagctacgtgtcctggtaccagcagctgcccggaaccgcccctaagctgctgatctacgacaacaacaagaggccctccggcgtgcccgacagatttagcggcagcaagagcggcaccagcgccacactggccatcacaggcctgcagaccggcgatgaggccgactactactgcggcacctgggacacaagccctgtgtgggaatggcccttcggcaccggcaccaagctgaccgtgctgaggaacgacgctcagccagccgtgtacctcttccagccttcgccggaccagcttcatacggggtcagcgtcggtggtgtgcctgttgaactcgttttaccccaaggacattaacgtgaagtggaaggtagacggggtaattcaagacactggcattcaagagtccgtcacggaacaagactcaaaagactcaacgtattcactgtcgtcaaccttgacgatgtcaagcaccgagtatcttagccatgagctgtattcgtgcgagatcacccacaagtccctcccctccactcttatcaaatcctttcagcggtcggaatgtcagcgggtcgat

SEQ ID NO: 22 - protein, 222 aa, Artificial Sequence
  Canis familiaris plus human
QSVLTQPPSVSAAPGQKVTISCSGGGSSIGNSYVSWYQQLPGTAPKLLIYDNNKRPSGVPDRFSGSKSGTSATLAITGLQTGDEADYYCGTWDTSPVWEWPFGTGTKLTVLRNDAQPAVYLFQPSPDQLHTGSASVVCLLNSFYPKDINVKWKVDGVIQDTGIQESVTEQDSKDSTYSLSSTLTMSSTEYLSHELYSCEITHKSLPSTLIKSFQRSECQRVD

SEQ ID NO: 23 - DNA, 1350 bp, Artificial Sequence
  Canis familiaris plus human
gaggtgcagctggtgcagagcggaggcggactggtgcatcccggaggaagcctgagactgtcctgcgccggcagcggcttcaccttcagcaggaacgccatgttctgggtgagacaggcccccggcaagggactggaatgggtgagcctgatcggaaccggaggcgccaccaactacgccgacagcgtgaagggcaggttcaccatcagcagggacaacgccaagaacagcctgtacctgcagatgaacagcctgagggccgaggacatggccgtgtactactgcgccaggggcaggtactacttcgactattggggccagggcaccctcgtgaccgtgtccagcgcttccacaaccgcgccatcagtctttccgttggccccatcatgcgggtcgacgagcggatcgactgtggccctggcgtgcttggtgtcgggatactttcccgaacccgtcacggtcagctggaactccggatcgcttacgagcggtgtgcatacgttcccctcggtcttgcaatcatcagggctctactcgctgtcgagcatggtaacggtgccctcatcgaggtggccctccgaaacgttcacatgtaacgtagcacatccagcctccaaaaccaaggtggataaacccgtgccgaaaagagagaatgggcgggtgcctcgaccccctgattgccccaagtgtccggctccggaaatgctcggtggaccctcagtgtttatcttccctccgaagcccaaggacactctgctgatcgcgcgcactccagaagtaacatgtgtagtggtggcacttgatcccgaggaccccgaagtccagatctcctggtttgtagatgggaaacagatgcagaccgcaaaaactcaacccagagaggagcagttcgcaggaacataccgagtggtatccgtccttccgattggccaccaggactggttgaaagggaagcagtttacgtgtaaagtcaacaataaggcgttgcctagccctattgagcggacgatttcgaaagctaggggacaggcccaccagccatcggtctatgtccttccgccttcccgcgaggagctctcgaagaatacagtgagccttacatgcctcattaaggatttcttcccgcctgatatcgacgtagagtggcaatcaaacggtcaacaggagccggaatccaagtatagaaccactccgccccagcttgacgaggacggatcatactttttgtattcaaaactgtcggtggataagagccggtggcagagaggtgacaccttcatctgtgcggtgatgcacgaagcactccataatcactacacccaagagagcctctcgcattcccccggaaag

SEQ ID NO: 24 - protein, 450 aa, Artificial Sequence
  Canis familiaris plus human
EVQLVQSGGGLVHPGGSLRLSCAGSGFTFSRNAMFWVRQAPGKGLEWVSLIGTGGATNYADSVKGRFTISRDNAKNSLYLQMNSLRAEDMAVYYCARGRYYFDYWGQGTLVTVSSASTTAPSVFPLAPSCGSTSGSTVALACLVSGYFPEPVTVSWNSGSLTSGVHTFPSVLQSSGLYSLSSMVTVPSSRWPSETFTCNVAHPASKTKVDKPVPKRENGRVPRPPDCPKCPAPEMLGGPSVFIFPPKPKDTLLIARTPEVTCVVVALDPEDPEVQISWFVDGKQMQTAKTQPREEQFAGTYRVVSVLPIGHQDWLKGKQFTCKVNNKALPSPIERTISKARGQAHQPSVYVLPPSREELSKNTVSLTCLIKDFFPPDIDVEWQSNGQQEPESKYRTTPPQLDEDGSYFLYSKLSVDKSRWQRGDTFICAVMHEALHNHYTQESLSHSPGK

SEQ ID NO: 25 - DNA, 660 bp, Artificial Sequence
  Canis familiaris plus human
gagatcgtgctgacccagagccctggcacactgagcctgagccccggagagagggctaccctgagctgcagggccagccagagcgtgagcagcagctacctggcctggtaccagcagaaacccggccaggcccccagactgctgatctttggcgccagcagcagagccaccggcatccccgatagatttagcggcagcggcagcggcaccgactttaccctgaccatcagcaggctggagcccgaggacttcgccgtgtactactgccagcagtacggcagcagccctccttggaccttcggccagggcaccaaggtggagatcaagaggaacgacgctcagccagccgtgtacctcttccagccttcgccggaccagcttcatacggggtcagcgtcggtggtgtgcctgttgaactcgttttaccccaaggacattaacgtgaagtggaaggtagacggggtaattcaagacactggcattcaagagtccgtcacggaacaagactcaaaagactcaacgtattcactgtcgtcaaccttgacgatgtcaagcaccgagtatcttagccatgagctgtattcgtgcgagatcacccacaagtccctcccctccactcttatcaaatcctttcagcggtcggaatgtcagcgggtcgat

SEQ ID NO: 26 - protein, 220 aa, Artificial Sequence
  Canis familiaris plus human
EIVLTQSPGTLSLSPGERATLSCRASQSVSSSYLAWYQQKPGQAPRLLIFGASSRATGIPDRFSGSGSGTDFTLTISRLEPEDFAVYYCQQYGSSPPWTFGQGTKVEIKRNDAQPAVYLFQPSPDQLHTGSASVVCLLNSFYPKDINVKWKVDGVIQDTGIQESVTEQDSKDSTYSLSSTLTMSSTEYLSHELYSCEITHKSLPSTLIKSFQRSECQRVD

SEQ ID NO: 27 - DNA, 1380 bp, Artificial Sequence
  Canis familiaris plus human
gaggtgcagctggtggagagcggcggagacctggtgaagcctggaggcagcctgagactgagctgcgtggccagcggcttcaccttcagggactacgccatgacctgggtgaggcaggctcctggaaagggcctgcagtgggtggcctccattagcggcagcggcggcaacacatactacgccgacagcgtgaagggcaggttcaccatcagcagggacaacgccaagaacaccctgtacctgcagatgaacagcctgagggccgaggacaccgccgtgtactactgcaccagggacaggctgtccatcaccatcaggcccaggtactacggcctggatgtgtggggccagggcacactggtgaccgtgagcagcgcttccacaaccgcgccatcagtctttccgttggccccatcatgcgggtcgacgagcggatcgactgtggccctggcgtgcttggtgtcgggatactttcccgaacccgtcacggtcagctggaactccggatcgcttacgagcggtgtgcatacgttcccctcggtcttgcaatcatcagggctctactcgctgtcgagcatggtaacggtgccctcatcgaggtggccctccgaaacgttcacatgtaacgtagcacatccagcctccaaaaccaaggtggataaacccgtgccgaaaagagagaatgggcgggtgcctcgaccccctgattgccccaagtgtccggctccggaaatgctcggtggaccctcagtgtttatcttccctccgaagcccaaggacactctgctgatcgcgcgcactccagaagtaacatgtgtagtggtggcacttgatcccgaggaccccgaagtccagatctcctggtttgtagatgggaaacagatgcagaccgcaaaaactcaacccagagaggagcagttcgcaggaacataccgagtggtatccgtccttccgattggccaccaggactggttgaaagggaagcagtttacgtgtaaagtcaacaataaggcgttgcctagccctattgagcggacgatttcgaaagctaggggacaggcccaccagccatcggtctatgtccttccgccttcccgcgaggagctctcgaagaatacagtgagccttacatgcctcattaaggatttcttcccgcctgatatcgacgtagagtggcaatcaaacggtcaacaggagccggaatccaagtatagaaccactccgccccagcttgacgaggacggatcatactttttgtattcaaaactgtcggtggataagagccggtggcagagaggtgacaccttcatctgtgcggtgatgcacgaagcactccataatcactacacccaagagagcctctcgcattcccccggaaag

SEQ ID NO: 28 - protein, 460 aa, Artificial Sequence
  Canis familiaris plus human
EVQLVESGGDLVKPGGSLRLSCVASGFTFRDYAMTWVRQAPGKGLQWVASISGSGGNTYYADSVKGRFTISRDNAKNTLYLQMNSLRAEDTAVYYCTRDRLSITIRPRYYGLDVWGQGTLVTVSSASTTAPSVFPLAPSCGSTSGSTVALACLVSGYFPEPVTVSWNSGSLTSGVHTFPSVLQSSGLYSLSSMVTVPSSRWPSETFTCNVAHPASKTKVDKPVPKRENGRVPRPPDCPKCPAPEMLGGPSVFIFPPKPKDTLLIARTPEVTCVVVALDPEDPEVQISWFVDGKQMQTAKTQPREEQFAGTYRVVSVLPIGHQDWLKGKQFTCKVNNKALPSPIERTISKARGQAHQPSVYVLPPSREELSKNTVSLTCLIKDFFPPDIDVEWQSNGQQEPESKYRTTPPQLDEDGSYFLYSKLSVDKSRWQRGDTFICAVMHEALHNHYTQESLSHSPGK

SEQ ID NO: 29 - DNA, 1380 bp, Artificial Sequence
  Canis familiaris plus human
gaggtgcagctggtggagagcggcggcgatctggtgaagcctggaggcagcctgagactgagctgcgccggaagcggcttcaccttcagggactacgccatgacctgggtgagacaggcccctggaaagggcctgcagtgggtgagcagcatctccggcagcggcggcaacacctactacgccgacagcgtgaagggcaggttcaccatcagcagggacaacgccaagaacaccctgtacctgcagatgaacagcctgagggccgaggacaccgccgtgtactactgcgccaaggacagactgagcatcaccatcaggcccaggtactacggcctggacgtgtggggacagggcacactggtgaccgtgagcagcgcttccacaaccgcgccatcagtctttccgttggccccatcatgcgggtcgacgagcggatcgactgtggccctggcgtgcttggtgtcgggatactttcccgaacccgtcacggtcagctggaactccggatcgcttacgagcggtgtgcatacgttcccctcggtcttgcaatcatcagggctctactcgctgtcgagcatggtaacggtgccctcatcgaggtggccctccgaaacgttcacatgtaacgtagcacatccagcctccaaaaccaaggtggataaacccgtgccgaaaagagagaatgggcgggtgcctcgaccccctgattgccccaagtgtccggctccggaaatgctcggtggaccctcagtgtttatcttccctccgaagcccaaggacactctgctgatcgcgcgcactccagaagtaacatgtgtagtggtggcacttgatcccgaggaccccgaagtccagatctcctggtttgtagatgggaaacagatgcagaccgcaaaaactcaacccagagaggagcagttcgcaggaacataccgagtggtatccgtccttccgattggccaccaggactggttgaaagggaagcagtttacgtgtaaagtcaacaataaggcgttgcctagccctattgagcggacgatttcgaaagctaggggacaggcccaccagccatcggtctatgtccttccgccttcccgcgaggagctctcgaagaatacagtgagccttacatgcctcattaaggatttcttcccgcctgatatcgacgtagagtggcaatcaaacggtcaacaggagccggaatccaagtatagaaccactccgccccagcttgacgaggacggatcatactttttgtattcaaaactgtcggtggataagagccggtggcagagaggtgacaccttcatctgtgcggtgatgcacgaagcactccataatcactacacccaagagagcctctcgcattcccccggaaag

SEQ ID NO: 30 - protein, 460 aa, Artificial Sequence
  Canis familiaris plus human
EVQLVESGGDLVKPGGSLRLSCAGSGFTFRDYAMTWVRQAPGKGLQWVSSISGSGGNTYYADSVKGRFTISRDNAKNTLYLQMNSLRAEDTAVYYCAKDRLSITIRPRYYGLDVWGQGTLVTVSSASTTAPSVFPLAPSCGSTSGSTVALACLVSGYFPEPVTVSWNSGSLTSGVHTFPSVLQSSGLYSLSSMVTVPSSRWPSETFTCNVAHPASKTKVDKPVPKRENGRVPRPPDCPKCPAPEMLGGPSVFIFPPKPKDTLLIARTPEVTCVVVALDPEDPEVQISWFVDGKQMQTAKTQPREEQFAGTYRVVSVLPIGHQDWLKGKQFTCKVNNKALPSPIERTISKARGQAHQPSVYVLPPSREELSKNTVSLTCLIKDFFPPDIDVEWQSNGQQEPESKYRTTPPQLDEDGSYFLYSKLSVDKSRWQRGDTFICAVMHEALHNHYTQESLSHSPGK

SEQ ID NO: 31 - DNA, 1380 bp, Artificial Sequence
  Canis familiaris plus human
gaggtgcagctggtggagagcggcggcgatctggtgaagcctggcggaagcctgagactgagctgtgccggcagcggcttcaccttcagggactacgccatgacctgggtgagacaggcccctggcaaaggcctggagtgggtgagcagcatcagcggcagcggcggcaacacctactacgccgacagcgtgaagggcaggttcaccatctccagggacaacagcaagaacaccctgtacctgcagatgaacagcctgagggccgaggataccgccgtgtactactgcgccaaggacagactgagcatcaccatcaggcccaggtactacggactggatgtgtggggccagggcaccctcgtgaccgtgtccagcgcttccacaaccgcgccatcagtctttccgttggccccatcatgcgggtcgacgagcggatcgactgtggccctggcgtgcttggtgtcgggatactttcccgaacccgtcacggtcagctggaactccggatcgcttacgagcggtgtgcatacgttcccctcggtcttgcaatcatcagggctctactcgctgtcgagcatggtaacggtgccctcatcgaggtggccctccgaaacgttcacatgtaacgtagcacatccagcctccaaaaccaaggtggataaacccgtgccgaaaagagagaatgggcgggtgcctcgaccccctgattgccccaagtgtccggctccggaaatgctcggtggaccctcagtgtttatcttccctccgaagcccaaggacactctgctgatcgcgcgcactccagaagtaacatgtgtagtggtggcacttgatcccgaggaccccgaagtccagatctcctggtttgtagatgggaaacagatgcagaccgcaaaaactcaacccagagaggagcagttcgcaggaacataccgagtggtatccgtccttccgattggccaccaggactggttgaaagggaagcagtttacgtgtaaagtcaacaataaggcgttgcctagccctattgagcggacgatttcgaaagctaggggacaggcccaccagccatcggtctatgtccttccgccttcccgcgaggagctctcgaagaatacagtgagccttacatgcctcattaaggatttcttcccgcctgatatcgacgtagagtggcaatcaaacggtcaacaggagccggaatccaagtatagaaccactccgccccagcttgacgaggacggatcatactttttgtattcaaaactgtcggtggataagagccggtggcagagaggtgacaccttcatctgtgcggtgatgcacgaagcactccataatcactacacccaagagagcctctcgcattcccccggaaag

SEQ ID NO: 32 - protein, 460 aa, Artificial Sequence
  Canis familiaris plus human
EVQLVESGGDLVKPGGSLRLSCAGSGFTFRDYAMTWVRQAPGKGLEWVSSISGSGGNTYYADSVKGRFTISRDNSKNTLYLQMNSLRAEDTAVYYCAKDRLSITIRPRYYGLDVWGQGTLVTVSSASTTAPSVFPLAPSCGSTSGSTVALACLVSGYFPEPVTVSWNSGSLTSGVHTFPSVLQSSGLYSLSSMVTVPSSRWPSETFTCNVAHPASKTKVDKPVPKRENGRVPRPPDCPKCPAPEMLGGPSVFIFPPKPKDTLLIARTPEVTCVVVALDPEDPEVQISWFVDGKQMQTAKTQPREEQFAGTYRVVSVLPIGHQDWLKGKQFTCKVNNKALPSPIERTISKARGQAHQPSVYVLPPSREELSKNTVSLTCLIKDFFPPDIDVEWQSNGQQEPESKYRTTPPQLDEDGSYFLYSKLSVDKSRWQRGDTFICAVMHEALHNHYTQESLSHSPGK

SEQ ID NO: 33 - DNA, 669 bp, Artificial Sequence
  Canis familiaris plus human
gacattgtgatgacccagacccctctgagcctgtccgtgagccctggcgagcctgctagcatcagctgcaggagcagccagagcctgctgtacagcatcggctacaactacctggactggttcaggcagaagcccggccagagccctcagaggctgatctacctgggaagcaacagggccagcggcgtgcctgacaggtttagcggcagcggcagcggcaccgatttcaccctgaggatcagcagagtggaggccgatgacgccggcgtgtactactgcatgcaggccctgcagaccccctacaccttcggccagggcaccaaggtggagatcaagaggaacgacgctcagccagccgtgtacctcttccagccttcgccggaccagcttcatacggggtcagcgtcggtggtgtgcctgttgaactcgttttaccccaaggacattaacgtgaagtggaaggtagacggggtaattcaagacactggcattcaagagtccgtcacggaacaagactcaaaagactcaacgtattcactgtcgtcaaccttgacgatgtcaagcaccgagtatcttagccatgagctgtattcgtgcgagatcacccacaagtccctcccctccactcttatcaaatcctttcagcggtcggaatgtcagcgggtcgat

SEQ ID NO: 34 - protein, 223 aa, Artificial Sequence
  Canis familiaris plus human
DIVMTQTPLSLSVSPGEPASISCRSSQSLLYSIGYNYLDWFRQKPGQSPQRLIYLGSNRASGVPDRFSGSGSGTDFTLRISRVEADDAGVYYCMQALQTPYTFGQGTKVEIKRNDAQPAVYLFQPSPDQLHTGSASVVCLLNSFYPKDINVKWKVDGVIQDTGIQESVTEQDSKDSTYSLSSTLTMSSTEYLSHELYSCEITHKSLPSTLIKSFQRSECQRVD

SEQ ID NO: 35 - DNA, 669 bp, Artificial Sequence
  Canis familiaris plus human
gacatcgtgatgacccagacccctctgagcctgagcgtgagccctggagagcccgccagcatctcctgcagaagcagccagagcctgctgtacagcatcggctacaactacctggactggtacctgcagaagcccggccagagccctcagctgctgatctacctgggcagcaacagagccagcggcgtgcctgacagatttagcggcagcggcagcggcacagacttcaccctgaggatcagcagagtggaggccgacgatgccggcgtgtactactgcatgcaggccctgcagaccccctacaccttcggccagggcaccaaggtggagatcaagaggaacgacgctcagccagccgtgtacctcttccagccttcgccggaccagcttcatacggggtcagcgtcggtggtgtgcctgttgaactcgttttaccccaaggacattaacgtgaagtggaaggtagacggggtaattcaagacactggcattcaagagtccgtcacggaacaagactcaaaagactcaacgtattcactgtcgtcaaccttgacgatgtcaagcaccgagtatcttagccatgagctgtattcgtgcgagatcacccacaagtccctcccctccactcttatcaaatcctttcagcggtcggaatgtcagcgggtcgat

SEQ ID NO: 36 - protein, 223 aa, Artificial Sequence
  Canis familiaris plus human
DIVMTQTPLSLSVSPGEPASISCRSSQSLLYSIGYNYLDWYLQKPGQSPQLLIYLGSNRASGVPDRFSGSGSGTDFTLRISRVEADDAGVYYCMQALQTPYTFGQGTKVEIKRNDAQPAVYLFQPSPDQLHTGSASVVCLLNSFYPKDINVKWKVDGVIQDTGIQESVTEQDSKDSTYSLSSTLTMSSTEYLSHELYSCEITHKSLPSTLIKSFQRSECQRVD

SEQ ID NO: 37 - DNA, 669 bp, Artificial Sequence
  Canis familiaris plus human
gacatcgtgatgacccagacacccctgagcctgagcgtgagccctggcgaacctgccagcatcagctgcaggagctcccagagcctgctgtacagcatcggctacaactacctcgactggtacctgcagaagcccggccagagccctcagctgctgatctacctgggctccaacagagccagcggcgtgcctgacagatttagcggcagcggcagcggaaccgacttcaccctgaggatcagcagagtggaggccgacgacgccggcttctactactgcatgcaggccctgcagaccccctacaccttcggccagggcaccaagctggagatcaagaggaacgacgctcagccagccgtgtacctcttccagccttcgccggaccagcttcatacggggtcagcgtcggtggtgtgcctgttgaactcgttttaccccaaggacattaacgtgaagtggaaggtagacggggtaattcaagacactggcattcaagagtccgtcacggaacaagactcaaaagactcaacgtattcactgtcgtcaaccttgacgatgtcaagcaccgagtatcttagccatgagctgtattcgtgcgagatcacccacaagtccctcccctccactcttatcaaatcctttcagcggtcggaatgtcagcgggtcgat

SEQ ID NO: 38 - protein, 223 aa, Artificial Sequence
  Canis familiaris plus human
DIVMTQTPLSLSVSPGEPASISCRSSQSLLYSIGYNYLDWYLQKPGQSPQLLIYLGSNRASGVPDRFSGSGSGTDFTLRISRVEADDAGFYYCMQALQTPYTFGQGTKLEIKRNDAQPAVYLFQPSPDQLHTGSASVVCLLNSFYPKDINVKWKVDGVIQDTGIQESVTEQDSKDSTYSLSSTLTMSSTEYLSHELYSCEITHKSLPSTLIKSFQRSECQRVD

SEQ ID NO: 39 - protein, 21 aa, Canis familiaris
QWKMDHPTNCSAELRLSYQLD

SEQ ID NO: 40 - protein, 11 aa, Canis familiaris
RLAASTLKSGA

SEQ ID NO: 41 - protein, 11 aa, Canis familiaris
TNCSAELRLSY

SEQ ID NO: 42 - protein, 4 aa, Canis familiaris
STLK

SEQ ID NO: 43 - protein, 16 aa, Homo sapiens
RSSQSLLYSIGYNYLD

SEQ ID NO: 44 - protein, 7 aa, Homo sapiens
LGSNRAS

SEQ ID NO: 45 - protein, 9 aa, Homo sapiens
MQALQTPYT

SEQ ID NO: 46 - protein, 5 aa, Homo sapiens
DYAMT

SEQ ID NO: 47 - protein, 17 aa, Homo sapiens
SISGSGGNTYYADSVKG

SEQ ID NO: 48 - protein, 16 aa, Homo sapiens
DRLSITIRPRYYGLDV

SEQ ID NO: 49 - protein, 13 aa, Homo sapiens
SGGGSSIGQSYVS

SEQ ID NO: 50 - protein, 7 aa, Homo sapiens
DNNKRPS

SEQ ID NO: 51 - protein, 12 aa, Homo sapiens
GTWDTSPVWEWP

SEQ ID NO: 52 - protein, 5 aa, Homo sapiens
SYYMH

SEQ ID NO: 53 - protein, 17 aa, Homo sapiens
IINPRGGSTSYAQKFQG

SEQ ID NO: 54 - protein, 7 aa, Homo sapiens
GKYWMYD

SEQ ID NO: 55 - protein, 12 aa, Homo sapiens
RASQSVSSSYLA

SEQ ID NO: 56 - protein, 7 aa, Homo sapiens
GASSRAT

SEQ ID NO: 57 - protein, 10 aa, Homo sapiens
QQYGSSPPWT

SEQ ID NO: 58 - protein, 5 aa, Homo sapiens
RNAMF

SEQ ID NO: 59 - protein, 16 aa, Homo sapiens
LIGTGGATNYADSVKG

SEQ ID NO: 60 - protein, 7 aa, Homo sapiens
GRYYFDY

SEQ ID NO: 61 - protein, 17 aa, Canis familiaris
FNECRCTDTPPCPVPEP

SEQ ID NO: 62 - protein, 22 aa, Canis familiaris
PKRENGRVPRPPDCPKCPAPEM

SEQ ID NO: 63 - protein, 20 aa, Canis familiaris
AKECECKCNCNNCPCPGCGL

SEQ ID NO: 64 - protein, 17 aa, Artificial Sequence
  modified canis famliaris
PKESTCKCIPPCPVPES

SEQ ID NO: 65 - protein, 13 aa, Homo sapiens
SGGSSNIGNSYVS

SEQ ID NO: 66 - protein, 7 aa, Homo sapiens
DNNKRPS

SEQ ID NO: 67 - protein, 12 aa, Homo sapiens
GTWDTSLSANYV

SEQ ID NO: 68 - protein, 5 aa, Homo sapiens
SYYMH

SEQ ID NO: 69 - protein, 17 aa, Homo sapiens
IINPSGGSTSYAQKFQG

SEQ ID NO: 70 - protein, 7 aa, Homo sapiens
GKWWLDY

SEQ ID NO: 71 - protein, 13 aa, Homo sapiens
SGGSSNIGNSYVS

SEQ ID NO: 72 - protein, 7 aa, Homo sapiens
DNNKRPS

SEQ ID NO: 73 - protein, 12 aa, Homo sapiens
GTWDTSTTMYPL

SEQ ID NO: 74 - protein, 5 aa, Homo sapiens
SYYMH

SEQ ID NO: 75 - protein, 17 aa, Homo sapiens
IINPSGGSTSYAQKFQG

SEQ ID NO: 76 - protein, 7 aa, Homo sapiens
GKWWFYD

SEQ ID NO: 77 - protein, 11 aa, Homo sapiens
RASQSVSSYLA

SEQ ID NO: 78 - protein, 7 aa, Homo sapiens
HASNRAT

SEQ ID NO: 79 - protein, 9 aa, Homo sapiens
QQRSNWPLT

SEQ ID NO: 80 - protein, 5 aa, Homo sapiens
NFVMH

SEQ ID NO: 81 - protein, 16 aa, Homo sapiens
AIGTGGGTYYADSVKG

SEQ ID NO: 82 - protein, 15 aa, Homo sapiens
DRPMVRGVIIDYFDY

SEQ ID NO: 83 - protein, 12 aa, Homo sapiens
RASQSVSSSYLA

SEQ ID NO: 84 - protein, 7 aa, Homo sapiens
GASSRAT

SEQ ID NO: 85 - protein, 10 aa, Homo sapiens
QQYGSSPPWT

SEQ ID NO: 86 - protein, 5 aa, Homo sapiens
RYGMH

SEQ ID NO: 87 - protein, 17 aa, Homo sapiens
IIWFEGNNQYYADSVKG

SEQ ID NO: 88 - protein, 7 aa, Homo sapiens
GKYYFDY

SEQ ID NO: 89 - protein, 11 aa, Homo sapiens
RASQGISTWLA

SEQ ID NO: 90 - protein, 7 aa, Homo sapiens
VASSLQS

SEQ ID NO: 91 - protein, 9 aa, Homo sapiens
QQANSFPFT

SEQ ID NO: 92 - protein, 5 aa, Homo sapiens
SYAMS

SEQ ID NO: 93 - protein, 17 aa, Homo sapiens
SITGSGGSTYYADSVKG

SEQ ID NO: 94 - protein, 8 aa, Homo sapiens
DNRGFFHY